European Patent Application EP 4 796 565 A1, published August 26, 2026. Title: 一种合成的抗癌脂肽及其应用. Applicant: 永州中古生物技术有限公司. Application CN. The sequence listing filed with the application follows.

SEQUENCE LISTING (3 sequences)

SEQ ID NO: 1 - protein, 25 aa, synthetic construct
  source 1..25: note = lipopeptide
  DISULFID 15..25: note = intrachain disulfide bond formed by Cys15 and Cys25
  LIPID 1: note = N-decanoyl glycine
  NON_STD 14: note = 3-amino propionic acid
  MOD_RES 25: note = amidation
GRKKRRQRRRPPQXCWMSPRHLGTC

SEQ ID NO: 2 - protein, 13 aa, synthetic construct
  source 1..13: note = X2 domain
GRKKRRQRRRPPQ

SEQ ID NO: 3 - protein, 11 aa, synthetic construct
  source 1..11: note = X3 domain
CWMSPRHLGTC